European Patent Specification EP 3 736 272 B1, published September 2, 2026. Title: Novel piperazine and piperidine derivatives, their synthesis and use thereof in inhibiting VDAC oligomerization, apoptosis and mitochondria dysfunction. Applicant: The National Institute for Biotechnology in the Negev Ltd. SHOSHAN-BARMATZ Varda GRUZMAN, Lev Arie. Application EP16845836.2. The sequence listing filed with the application follows.

SEQUENCE LISTING (4 sequences)

SEQ ID NO: 1 - DNA, 32 bp, Artificial Sequence
  rVDAC1 forward primer
cgaagcttatggctgtgccacccacgtatgcc

SEQ ID NO: 2 - DNA, 42 bp, Artificial Sequence
  rVDAC reverse primer
ggatccgccgccgccggagccgccgccgcctgcttgaaattc

SEQ ID NO: 3 - DNA, 57 bp, Artificial Sequence
  encoding shRNA against hVDAC1 targeting sequence
agcttaaaaacactaggcaccgagattatctcttgaataatctcggtgcctagtgtg

SEQ ID NO: 4 - DNA, 58 bp, Artificial Sequence
  encoding shRNA against hVDAC1 anti-sense sequence
gatccacactaggcaccgagattattcaagagataatctcggtgcctagtgtttttta